European Patent Application EP 4 741 498 A1, published May 13, 2026. Title: 一种免疫球蛋白降解酶IdeE的突变体. Applicant: 上海宝济药业股份有限公司. Application CN. The sequence listing filed with the application follows.

SEQUENCE LISTING (3 sequences)

SEQ ID NO: 1 - protein, 297 aa, synthetic construct
ITSVWTKGVTPLTPEQFRYNNEDVIHAPYLAHQGWYDITKAFDGKDNLLCGAATAGNMLHWWFDQNKTEIEAYLSKHPDKQKIIFNNQELFDLKAAIDTKDSQTNSQLFNYFRDKAFPNLSARQLGVMPDLVLDMFINGYYLNVFKTQSTDVNRPYQDKDKRGGIFDAVFTRGDQTTLLTARHDLKNKGLNDISTIIKQELTEGRALALSHTYANVSISHVINLWGADFNAEGNLEAIYVTDSDANASIGMKKYFVGINAHGHVAISAKKIEGENIGAQVLGLFTLSSGKDIWQKLS

SEQ ID NO: 2 - protein, 298 aa, synthetic construct
MITSVWTKGVTPLTPEQFRYNNEDVIHAPYLAHQGWYDITKAFDGKDNLLCGAATAGNMLHWWFDQNKTEIEAYLSKHPDKQKIIFNNQELFDLKAAIDTKDSQTNSQLFNYFRDKAFPNLSARQLGVMPDLVLDMFINGYYLNVFKTQSTDVNRPYQDKDKRGGIFDAVFTRGDQTTLLTARHDLKNKGLNDISTIIKQELTEGRALALSHTYANVSISHVINLWGADFNAEGNLEAIYVTDSDANASIGMKKYFVGINAHGHVAISAKKIEGENIGAQVLGLFTLSSGKDIWQKLS

SEQ ID NO: 3 - DNA, 900 bp, synthetic construct
  source 1..900: mol_type = other DNA
atgatcaccagcgtgtggaccaaaggtgttaccccgctgaccccggagcagttccgttacaacaacgaagacgttattcacgcgccgtacctggcgcaccaaggttggtatgatatcaccaaggcgttcgacggcaaagataacctgctgtgcggtgcggcgaccgcgggtaacatgctgcactggtggtttgaccagaacaagaccgagattgaagcgtacctgagcaaacacccggataagcagaagatcatcttcaacaaccaagaactgttcgacctgaaggcggcgatcgacaccaaagatagccagaccaacagccaactgttcaactattttcgtgataaggcgtttccgaacctgagcgcgcgtcagctgggtgtgatgccggacctggttctggatatgttcattaacggctactatctgaacgtgtttaaaacccagagcaccgatgttaaccgtccgtaccaagacaaggataaacgtggtggcatcttcgacgcggtgtttacccgtggtgatcagaccaccctgctgaccgcgcgtcacgacctgaagaacaaaggtctgaacgatattagcaccatcattaagcaagaactgaccgaaggtcgtgcgctggcgctgagccacacctatgcgaacgtgagcatcagccacgttattaacctgtggggtgcggacttcaacgcggagggcaacctggaagcgatctacgtgaccgacagcgatgcgaacgcgagcattggcatgaagaaatattttgtgggtatcaacgcgcacggccacgttgcgatcagcgcgaagaaaattgagggtgaaaacatcggcgcgcaggttctgggtctgttcaccctgagcagcggcaaggatatttggcaaaaactgagctaatga